European Patent Application EP 4 163 365 A1, published April 12, 2023. Title: Method of producing cardiomyocyte population, method of proliferating cardiomyocytes, cardiomyocyte population, transplantation material, multinucleated cardiomyocyte, and kit for proliferating cardiomyocytes. Applicant: Myoridge Co. Ltd. The sequence listing filed with the application follows.

SEQUENCE LISTING (4 sequences)

SEQ ID NO: 1 - DNA, 17 bp, Artificial Sequence
  Forward primer for Lin28
cacggtgcgggcatctg

SEQ ID NO: 2 - DNA, 21 bp, Artificial Sequence
  Reverse primer for Lin28
ccttccatgtgcagcttactc

SEQ ID NO: 3 - DNA, 22 bp, Artificial Sequence
  Forward primer for cTnT
gaaggacctgaatgagttgcag

SEQ ID NO: 4 - DNA, 23 bp, Artificial Sequence
  Reverse primer for cTnT
acgtsctctcgatcctgtctttg